European Patent Application EP 4 640 233 A1, published October 29, 2025. Title: Hydrogel Preparations for Acute and Chronic Wound Healing. Applicant: UAB Bioremedium. The sequence listing filed with the application follows.

SEQUENCE LISTING (1 sequence)

SEQ ID NO: 1 - protein, 399 aa, Homo sapiens
EPAVYFKEQFLDGDGWTSRWIESKHKSDFGKFVLSSGKFYGDEEKDKGLQTSQDARFYALSASFEPFSNKGQTLWQFTVKHEQNIDCGGGYVKLFPNSLDQTDMHGDSEYNIMFGPDICGPGTKKVHVIFNYKGKNVLINKDIRCKDDEFTHLYTLIVRPDNTYEVKIDNSQVESGSLEDDWDFLPPKKIKDPDASKPEDWDERAKIDDPTDSKPEDWDKPEHIPDPDAKKPEDWDEEMDGEWEPPVIQNPEYKGEWKPRQIDNPDYKGTWIHPEIDNPEYSPDPSIYAYDNFGVLGLDLWQVKSGTIFDNFLITNDEAYAEEFGNETWGVTKAAEKQMKDKQDEEQRLKEEEEDKKRKEEEEAEDKEDDEDKDEDEEDEEDKEEDEEEDVPGQAKDEL